European Patent Application EP 4 368 189 A1, published May 15, 2024. Title: Peptides and combinations of peptides for use in immunotherapy against acute myeloid leukemia (AML) and other hematological neoplasms. Applicant: Eberhard Karls Universität Tübingen - Medizinische Fakultät. Application EP. The sequence listing filed with the application follows.

SEQUENCE LISTING (41 sequences)

SEQ ID NO: 1 - protein, 22 aa, synthetic construct
KLKKMWKSPNGTIQNILGGTVF

SEQ ID NO: 2 - protein, 16 aa, synthetic construct
DRVKLGTDYRLHLSPV

SEQ ID NO: 3 - protein, 16 aa, synthetic construct
ETLHKFASKPASEFVK

SEQ ID NO: 4 - protein, 22 aa, synthetic construct
PHRKKKPFIEKKKAVSFHLVHR

SEQ ID NO: 5 - protein, 16 aa, synthetic construct
SPGPFPFIQDNISFYA

SEQ ID NO: 6 - protein, 14 aa, synthetic construct
IGSYIERDVTPAIM

SEQ ID NO: 7 - protein, 15 aa, synthetic construct
SKPGVIFLTKKGRRF

SEQ ID NO: 8 - protein, 16 aa, synthetic construct
DRQQMEALTRYLRAAL

SEQ ID NO: 9 - protein, 15 aa, synthetic construct
GNQLFRINEANQLMQ

SEQ ID NO: 10 - protein, 17 aa, synthetic construct
LGQEVALNANTKNQKIR

SEQ ID NO: 11 - protein, 14 aa, synthetic construct
NGRTFHLTRTLTVK

SEQ ID NO: 12 - protein, 16 aa, synthetic construct
LDTMRQIQVFEDEPAR

SEQ ID NO: 13 - protein, 15 aa, synthetic construct
VVGYALDYNEYFRDL

SEQ ID NO: 14 - protein, 16 aa, synthetic construct
KHLHYWFVESQKDPEN

SEQ ID NO: 15 - protein, 13 aa, synthetic construct
ERPEWIHVDSRPF

SEQ ID NO: 16 - protein, 9 aa, synthetic construct
AVEEVSLRK

SEQ ID NO: 17 - protein, 9 aa, synthetic construct
LAVEEVSLR

SEQ ID NO: 18 - protein, 9 aa, synthetic construct
SLLEADPFL

SEQ ID NO: 19 - protein, 9 aa, synthetic construct
IILDALPQL

SEQ ID NO: 20 - protein, 9 aa, synthetic construct
ILNDVAMFL

SEQ ID NO: 21 - protein, 9 aa, synthetic construct
DIDTRSEFY

SEQ ID NO: 22 - protein, 9 aa, synthetic construct
FSEYFGAIY

SEQ ID NO: 23 - protein, 10 aa, synthetic construct
YLDGRLEPLY

SEQ ID NO: 24 - protein, 10 aa, synthetic construct
APESKHKSSL

SEQ ID NO: 25 - protein, 8 aa, synthetic construct
APGLHLEL

SEQ ID NO: 26 - protein, 10 aa, synthetic construct
APTIVGKSSL

SEQ ID NO: 27 - protein, 9 aa, synthetic construct
AYHELAQVY

SEQ ID NO: 28 - protein, 8 aa, synthetic construct
SRPPLLGF

SEQ ID NO: 29 - protein, 9 aa, synthetic construct
IYSGYIFDY

SEQ ID NO: 30 - protein, 8 aa, synthetic construct
DLDTRVAL

SEQ ID NO: 31 - protein, 10 aa, synthetic construct
APTPRIKAEL

SEQ ID NO: 32 - protein, 9 aa, synthetic construct
EGYGRYLDL

SEQ ID NO: 33 - protein, 9 aa, synthetic construct
GSEELRSLY

SEQ ID NO: 34 - protein, 9 aa, synthetic construct
YLLPAIVHI

SEQ ID NO: 35 - protein, 9 aa, synthetic construct
RLRPGGKKK

SEQ ID NO: 36 - protein, 10 aa, synthetic construct
TPGPGVRYPL

SEQ ID NO: 37 - protein, 8 aa, synthetic construct
DIAARNVL

SEQ ID NO: 38 - protein, 10 aa, synthetic construct
ASEDYVAPPK

SEQ ID NO: 39 - protein, 15 aa, synthetic construct
ETVITVDTKAAGKGK

SEQ ID NO: 40 - protein, 10 aa, synthetic construct
ILLSPPLLTI

SEQ ID NO: 41 - protein, 9 aa, synthetic construct
GPDDGRGVL